European Patent Specification EP 3 362 562 B1, published July 22, 2026. Title: ANTISENSE OLIGONUCLEOTIDES FOR USE IN TREATING ALZHEIMER'S DISEASE. Applicant: Academisch Ziekenhuis Leiden, also acting under the name Leiden University Medical Centre (LUMC). Application EP 16782057.0. The sequence listing filed with the application follows.

SEQUENCE LISTING (60 sequences)

SEQ ID NO: 1 - RNA, 251 nt, Homo sapiens
  intron 16 - exon 17 - intron 17
auuauauugcauuuagaaauuaaaauucuuuuucuuaauuuguuuucaagguguucuuugcagaagauguggguucaaacaaaggugcaaucauuggacucauggugggcgguguugucauagcgacagugaucgucaucaccuuggugaugcugaagaagaaacaguacacauccauucaucauggugugguggagguagguaaacuugacugcauguuuccaagugggaauuaagacuaugagagaauu

SEQ ID NO: 2 - protein, 14 aa, Homo sapiens
  C-terminal portion of the A-beta peptide
GAIIGLMVGGVVIA

SEQ ID NO: 3 - RNA, 147 nt, Homo sapiens
  Exon 17
guguucuuugcagaagauguggguucaaacaaaggugcaaucauuggacucauggugggcgguguugucauagcgacagugaucgucaucaccuuggugaugcugaagaagaaacaguacacauccauucaucauggugugguggag

SEQ ID NO: 4 - protein, 646 aa, Homo sapiens
  APP646
MLPGLALLLLAAWTARALEVPTDGNAGLLAEPQIAMFCGRLNMHMNVQNGKWDSDPSGTKTCIDTKEGILQYCQEVYPELQITNVVEANQPVTIQNWCKRGRKQCKTHPHFVIPYRCLVGEFVSDALLVPDKCKFLHQERMDVCETHLHWHTVAKETCSEKSTNLHDYGMLLPCGIDKFRGVEFVCCPLAEESDNVDSADAEEDDSDVWWGGADTDYADGSEDKVVEVAEEEEVAEVEEEEADDDEDDEDGDEVEEEAEEPYEEATERTTSIATTTTTTTESVEEVVRVPTTAASTPDAVDKYLETPGDENEHAHFQKAKERLEAKHRERMSQVMREWEEAERQAKNLPKADKKAVIQHFQEKVESLEQEAANERQQLVETHMARVEAMLNDRRRLALENYITALQAVPPRPRHVFNMLKKYVRAEQKDRQHTLKHFEHVRMVDPKKAAQIRSQVMTHLRVIYERMNQSLSLLYNVPAVAEEIQDEVDELLQKEQNYSDDVLANMISEPRISYGNDALMPSLTETKTTVELLPVNGEFSLDDLQPWHSFGADSVPANTENEVEPVDARPAADRGLTTRPGSGLTNIKTEEISEVKMDAEFRHDSGYEVHHQKLVDAAVTPEERHLSKMQQNGYENPTYKFFEQMQN

SEQ ID NO: 5 - protein, 695 aa, Homo sapiens
  APP695
MLPGLALLLLAAWTARALEVPTDGNAGLLAEPQIAMFCGRLNMHMNVQNGKWDSDPSGTKTCIDTKEGILQYCQEVYPELQITNVVEANQPVTIQNWCKRGRKQCKTHPHFVIPYRCLVGEFVSDALLVPDKCKFLHQERMDVCETHLHWHTVAKETCSEKSTNLHDYGMLLPCGIDKFRGVEFVCCPLAEESDNVDSADAEEDDSDVWWGGADTDYADGSEDKVVEVAEEEEVAEVEEEEADDDEDDEDGDEVEEEAEEPYEEATERTTSIATTTTTTTESVEEVVRVPTTAASTPDAVDKYLETPGDENEHAHFQKAKERLEAKHRERMSQVMREWEEAERQAKNLPKADKKAVIQHFQEKVESLEQEAANERQQLVETHMARVEAMLNDRRRLALENYITALQAVPPRPRHVFNMLKKYVRAEQKDRQHTLKHFEHVRMVDPKKAAQIRSQVMTHLRVIYERMNQSLSLLYNVPAVAEEIQDEVDELLQKEQNYSDDVLANMISEPRISYGNDALMPSLTETKTTVELLPVNGEFSLDDLQPWHSFGADSVPANTENEVEPVDARPAADRGLTTRPGSGLTNIKTEEISEVKMDAEFRHDSGYEVHHQKLVFFAEDVGSNKGAIIGLMVGGVVIATVIVITLVMLKKKQYTSIHHGVVEVDAAVTPEERHLSKMQQNGYENPTYKFFEQMQN

SEQ ID NO: 6 - protein, 49 aa, Homo sapiens
  Skipped sequence (aa.608-656 of SEQ ID NO: 5)
VFFAEDVGSNKGAIIGLMVGGVVIATVIVITLVMLKKKQYTSIHHGVVE

SEQ ID NO: 7 - DNA, 22 bp, Artificial Sequence
  Forward primer
tccgacatgactcaggatatga

SEQ ID NO: 8 - DNA, 20 bp, Artificial Sequence
  Reverse primer
tagccgttctgctgcatctt

SEQ ID NO: 9 - RNA, 22 nt, Artificial Sequence
  Antisense oligonucleotide AON1
uucugcaaagaacaccuugaaa

SEQ ID NO: 10 - RNA, 22 nt, Artificial Sequence
  Antisense oligonucleotide AON2
accuuucuuugaacccacaucu

SEQ ID NO: 11 - RNA, 24 nt, Artificial Sequence
  Antisense oligonucleotide AON3
aaugauugcaccuuuguuugaacc

SEQ ID NO: 12 - RNA, 21 nt, Artificial Sequence
  Antisense oligonucleotide AON4
cgcccaccaugaguccaauga

SEQ ID NO: 13 - RNA, 20 nt, Artificial Sequence
  Antisense oligonucleotide AON5
acugucgcuaugacaacacc

SEQ ID NO: 14 - RNA, 20 nt, Artificial Sequence
  Antisense oligonucleotide AON6
uguacuguuucuucuucagc

SEQ ID NO: 15 - RNA, 20 nt, Artificial Sequence
  Antisense oligonucleotide AON7
gaugaauggauguguacugu

SEQ ID NO: 16 - RNA, 22 nt, Artificial Sequence
  Antisense oligonucleotide AON8
ucaaguuuaccuaccuccacca

SEQ ID NO: 17 - RNA, 24 nt, Artificial Sequence
  Antisense oligonucleotide AON1-1
gaacaccuugaaaacaaauuaaga

SEQ ID NO: 18 - RNA, 25 nt, Artificial Sequence
  Antisense oligonucleotide AON1-2
acaucuucugcaaagaacaccuuga

SEQ ID NO: 19 - RNA, 25 nt, Artificial Sequence
  Antisense oligonucleotide AON1-3
uucugcaaagaacaccuugaaaaca

SEQ ID NO: 20 - RNA, 31 nt, Artificial Sequence
  Antisense oligonucleotide AON1-4
aucuucugcaaagcaacaccuugaaaacaaa

SEQ ID NO: 21 - RNA, 20 nt, Artificial Sequence
  hAPPEx16_1 (LUMC1)
accaugaguccaaugauugc

SEQ ID NO: 22 - RNA, 20 nt, Artificial Sequence
  hAPPEx16_2 (LUMC2)
ucaccaaggugaugacgauc

SEQ ID NO: 23 - RNA, 23 nt, Artificial Sequence
  hAPPEx16_3 (LUMC3)
caccaugaugaauggauguguac

SEQ ID NO: 24 - RNA, 21 nt, Artificial Sequence
  hAPPEx16_4 (LUMC4)
guuugaacccacaucuucugc

SEQ ID NO: 25 - RNA, 22 nt, Artificial Sequence
  hAPPEx16_5 (LUMC5)
cuguuucuucuucagcaucacc

SEQ ID NO: 26 - RNA, 23 nt, Artificial Sequence
  hAPPEx16_6 (LUMC6)
cuaccuccaccacaccaugauga

SEQ ID NO: 27 - DNA, 42 bp, Artificial Sequence
  OL-1 DNA mouse
  /note="Combined DNA / RNA"
ggcgcctttgttcgaacccacaucttcagcaaagaacaccag

SEQ ID NO: 28 - RNA, 42 nt, Artificial Sequence
  OL-1 RNA mouse
ggcgccuuuguucgaacccacaucuucagcaaagaacaccag

SEQ ID NO: 29 - RNA, 42 nt, Artificial Sequence
  OL-1 hRNA / HOL1-RNA
ugcaccuuuguuugaacccacaucuucugcaaagaacaccuu

SEQ ID NO: 30 - RNA, 14 nt, Artificial Sequence
  OL-3
aacccacaucuuca

SEQ ID NO: 31 - RNA, 57 nt, Homo sapiens
  Part of exon 17 of the human APP gene
ucuuaauuuguuuucaagguguucuuugcagaagauguggguucaaacaaaggugca

SEQ ID NO: 32 - RNA, 15 nt, Homo sapiens
  Part of exon 17 of the human APP gene
guguucuuugcagaa

SEQ ID NO: 33 - RNA, 16 nt, Homo sapiens
  Part of exon 17 of the human APP gene
guguucuuugcagaag

SEQ ID NO: 34 - RNA, 17 nt, Homo sapiens
  Part of exon 17 of the human APP gene
guguucuuugcagaaga

SEQ ID NO: 35 - RNA, 18 nt, Homo sapiens
  Part of exon 17 of the human APP gene
guguucuuugcagaagau

SEQ ID NO: 36 - RNA, 36 nt, Homo sapiens
  Part of intron16/exon17 of the human APP gene
ucuuaauuuguuuucaagguguucuuugcagaagau

SEQ ID NO: 37 - RNA, 39 nt, Artificial Sequence
  QRX-203h (39)
accuuuguuugaacccacaucuucugcaaagaacaccuu

SEQ ID NO: 38 - RNA, 36 nt, Artificial Sequence
  QRX-203h (36)
uuuguuugaacccacaucuucugcaaagaacaccuu

SEQ ID NO: 39 - RNA, 33 nt, Artificial Sequence
  QRX-203h (33)
guuugaacccacaucuucugcaaagaacaccuu

SEQ ID NO: 40 - RNA, 30 nt, Artificial Sequence
  QRX-203h (30)
ugaacccacaucuucugcaaagaacaccuu

SEQ ID NO: 41 - RNA, 27 nt, Artificial Sequence
  QRX-203h (27)
acccacaucuucugcaaagaacaccuu

SEQ ID NO: 42 - RNA, 39 nt, Artificial Sequence
  QRX-203m (39)
gccuuuguucgaacccacaucuucagcaaagaacaccuu

SEQ ID NO: 43 - RNA, 36 nt, Artificial Sequence
  QRX-203m (36)
uuuguucgaacccacaucuucagcaaagaacaccuu

SEQ ID NO: 44 - RNA, 33 nt, Artificial Sequence
  QRX-203m (33)
guucgaacccacaucuucagcaaagaacaccuu

SEQ ID NO: 45 - RNA, 30 nt, Artificial Sequence
  QRX-203m (30)
cgaacccacaucuucagcaaagaacaccuu

SEQ ID NO: 46 - RNA, 27 nt, Artificial Sequence
  QRX-203m (27)
acccacaucuucagcaaagaacaccuu

SEQ ID NO: 47 - RNA, 26 nt, Artificial Sequence
  AON1-2-1
ccacaucuucugcaaagaacaccuug

SEQ ID NO: 48 - RNA, 30 nt, Artificial Sequence
  AON1-4-1
aucuucugcaaagaacaccuugaaaacaaa

SEQ ID NO: 49 - RNA, 34 nt, Artificial Sequence
  AON1-4-2
ccacaucuucugcaaagaacaccuugaaaacaaa

SEQ ID NO: 50 - DNA, 20 bp, Artificial Sequence
  Forward primer
tctgggctgacaaacatcaa

SEQ ID NO: 51 - DNA, 20 bp, Artificial Sequence
  Reverse primer
ttctgctgcatcttggagag

SEQ ID NO: 52 - protein, 75 aa, Homo sapiens
  Exon 16 - Exon 17 - Exon 18 of APP
DAEFRHDSGYEVHHQKLVFFAEDVGSNKGAIIGLMVGGVVIATVIVITLVMLKKKQYTSIHHGVVEVDAAVTPEE

SEQ ID NO: 53 - protein, 26 aa, Homo sapiens
  Exon 16 - Exon 18 of APP
DAEFRHDSGYEVHHQKLVDAAVTPEE

SEQ ID NO: 54 - protein, 14 aa, Homo sapiens
  APP
TEEISEVKMDAEFR

SEQ ID NO: 55 - protein, 5 aa, Homo sapiens
  APP
HQKLV

SEQ ID NO: 56 - protein, 5 aa, Homo sapiens
  APP
VGSNK

SEQ ID NO: 57 - protein, 15 aa, Homo sapiens
  APP
TVIVITLVMLKKKQY

SEQ ID NO: 58 - protein, 5 aa, Homo sapiens
  APP
EQMQN

SEQ ID NO: 59 - protein, 34 aa, Homo sapiens
  APP
VGSNKGAIIGLMVGGVVIATVIVITLVMLKKKQY

SEQ ID NO: 60 - RNA, 199 nt, Homo sapiens
  exon 17 of human APP and flanking regions
cuuuuucuuaauuuguuuucaagguguucuuugcagaagauguggguucaaacaaaggugcaaucauuggacucauggugggcgguguugucauagcgacagugaucgucaucaccuuggugaugcugaagaagaaacaguacacauccauucaucauggugugguggagguagguaaacuugacugcauguuuccaag